European Patent Application EP 4 692 292 A1, published February 11, 2026. Title: Improved method for germinating bacterial spores. Applicant: Evonik Operations GmbH. Application EP. The sequence listing filed with the application follows.

SEQUENCE LISTING (29 sequences)

SEQ ID NO: 1 - DNA, 1550 bp, Bacillus velezensis
  source 1..1550: mol_type = genomic DNA
ttatcggagagtttgatcctggctcaggacgaacgctggcggcgtgcctaatacatgcaagtcgagcggacagatgggagcttgctccctgatgttagcggcggacgggtgagtaacacgtgggtaacctgcctgtaagactgggataactccgggaaaccggggctaataccggatggttgtttgaaccgcatggttcagacataaaaggtggcttcggctaccacttacagatggacccgcggcgcattagctagttggtgaggtaacggctcaccaaggcgacgatgcgtagccgacctgagagggtgatcggccacactgggactgagacacggcccagactcctacgggaggcagcagtagggaatcttccgcaatggacgaaagtctgacggagcaacgccgcgtgagtgatgaaggttttcggatcgtaaagctctgttgttagggaagaacaagtgccgttcaaatagggcggcaccttgacggtacctaaccagaaagccacggctaactacgtgccagcagccgcggtaatacgtaggtggcaagcgttgtccggaattattgggcgtaaagggctcgcaggcggtttcttaagtctgatgtgaaagcccccggctcaaccggggagggtcattggaaactggggaacttgagtgcagaagaggagagtggaattccacgtgtagcggtgaaatgcgtagagatgtggaggaacaccagtggcgaaggcgactctctggtctgtaactgacgctgaggagcgaaagcgtggggagcgaacaggattagataccctggtagtccacgccgtaaacgatgagtgctaagtgttagggggtttccgccccttagtgctgcagctaacgcattaagcactccgcctggggagtacggtcgcaagactgaaactcaaaggaattgacgggggcccgcacaagcggtggagcatgtggtttaattcgaagcaacgcgaagaaccttaccaggtcttgacatcctctgacaatcctagagataggacgtccccttcgggggcagagtgacaggtggtgcatggttgtcgtcagctcgtgtcgtgagatgttgggttaagtcccgcaacgagcgcaacccttgatcttagttgccagcattcagttgggcactctaaggtgactgccggtgacaaaccggaggaaggtggggatgacgtcaaatcatcatgccccttatgacctgggctacacacgtgctacaatggacagaacaaagggcagcgaaaccgcgaggttaagccaatcccacaaatctgttctcagttcggatcgcagtctgcaactcgactgcgtgaagctggaatcgctagtaatcgcggatcagcatgccgcggtgaatacgttcccgggccttgtacacaccgcccgtcacaccacgagagtttgtaacacccgaagtcggtgaggtaaccttttaggagccagccgccgaaggtgggacagatgattggggtgaagtcgtaacaaggtagccgtatcggaaggtgcggctggatcacctccttt

SEQ ID NO: 2 - DNA, 3582 bp, Bacillus velezensis
  source 1..3582: mol_type = genomic DNA
ttgacaggtcaactagttcagtatggacgacaccgccagcgcagaagctatgctcgcattagcgaagtgttagaattaccaaatctcattgaaattcaaacctcttcttatcagtggtttcttgatgagggtcttagagagatgtttcaagacatatcaccaattgaggatttcactggtaacctctctctagagttcattgactacagtttaggagatcctaagtatcccgttgaagagtcaaaagaacgtgatgtgacttactcagctccgctgagagtgaaggttcgtttaattaacaaagaaactggagaggtaaaagaccaggatgtcttcatgggtgatttccctattatgacagataccggtacttttatcatcaacggtgcagaacgtgttatcgtatctcagcttgttcggtctccaagtgtatatttcagtggtaaagtagacaagaacggtaaaaaaggttttaccgcgactgtcattccaaaccgtggcgcatggttagaatacgaaactgatgcgaaagatgttgtgtatgtccgcattgatcgcacacgtaagttgccggttacggttcttttgcgtgctctcggcttcggttccgaccaagagattctcgatctcattggtgagaacgaatatctccgcaatacactggataaggacaacactgaaaacagtgacaaagcgcttcttgaaatctatgagcgccttcgtcccggagagccgcctacagtagaaaacgcaaaaagcttgctggattcccgtttcttcgatccgaagcgatacgaccttgcgaatgtaggacgctataaaattaataaaaagcttcatatcaagaaccgcctgtttaaccagcgccttgcagaaacactggtggatccggaaaccggtgaaattctcgctgaaaaagggcagattcttgacagaagaacacttgataaagtactgccatacttagaaaatggaatcggcttcagaaagctttatcctaacggcggcgttgtcgaggatgaagtgatgcttcaatccattaaaatctatgctcctaccgatgcagaaggagagcagacgatcaatgtgatcggcaatgcttacatcgaagaggcgattaaaaacattacgcctgctgatattatttcttctatcagctacttcttcaacctcctgcacggagtgggcgacactgatgatatcgaccatctcggaaaccgccgtctgcgttctgtaggtgagctcctgcaaaaccaattccgtatcggtttaagccggatggaacgtgtcgtacgtgaaagaatgtctattcaagacacgaatacaattacgccgcagcagctgattaacatcagacctgttattgcgtctattaaagagttcttcggaagctcacagctttctcaattcatggatcagacgaacccgcttgctgaattgacgcacaaacgccgtctgtcagctctcggaccgggcggtttgacacgtgagcgcgcaggtatggaagtacgtgacgttcactactctcactatggccgtatgtgtccgattgaaacgcctgagggcccgaacatcggtttgatcaactcattgtcatcatttgcgaaagtaaaccgctttggtttcattgagacgccataccgccgcgttgatcctgaaacaggaaaagtaacgcctagaatcgactacctgactgctgatgaagaggataactatgtcgtagcccaagcgaatgctaagctgagcgatgacggttctttcttggatgacagcatcgtagcgcgtttcagaggggaaaacaccgttgtagcccgcaaccgcgtggattacatggacgtatctcctaaacaggttgtatctgctgcgacagcatgtattccgttcttggaaaacgatgactcgaaccgtgccctcatgggagcgaacatgcagcgtcaggctgtgcctttgatgcagccggaagctccgatcgtcggaacgggtatggaatacgtatccggtaaagactccggtgcagccgttatttgtaaacaccctggtatcgttgaacgggtggaagcgaaaaacgtatgggtgcgccgctatgaagaaattgacggccaaaaagtaaaaggcaacctggataagtacagcttgctgaaatttgtccgctccaaccaaggtacgtgctacaaccagcgtccgatcgtcagtgtcggcgatgaagtagtcaaaggagaaatccttgctgacggaccttcaatggagcttggtgaacttgctctcggccgcaacgtaatggtcggcttcatgacatgggatggttacaactatgaggatgccatcatcatgagtgaacgccttgtgaaagatgatgtatacacatctattcacattgaagaatatgaatcagaagcacgtgatacaaagcttgggccggaagagatcacccgcgatattccaaacgtaggggaagacgcgcttcgcaatcttgatgaccgcggaattatccgtatcggtgcggaagtcaacgacggagaccttctcgtaggtaaagtaacgcctaaaggtgtaactgagcttacggctgaagaacgccttctgcatgcgatctttggagaaaaagcgcgtgaagtccgtgatacttctctccgtgtgcctcacggcggcggcggaattatccacgacgtaaaagtcttcaaccgtgaagacggcgacgaacttcctccgggagtgaaccagcttgtacgcgtatatatcgttcagaaacgtaagatttctgaaggtgataaaatggccggacgtcacggaaacaaaggggttatctcgaagattcttcctgaagaagatatgccttaccttcctgacggcacgccgatcgatatcatgcttaacccgctgggtgtaccatcacgtatgaatatcggtcaggtattagaacttcacatgggtatggctgcccgctacctcggcattcacatcgcgtcacctgtatttgacggcgcgcgtgaagaagatgtgtgggaaacacttgaagaagcaggcatgtcaagagacgctaaaacagttctttatgacggccgtacgggtgaaccgtttgacaaccgtgtatctgtcggaatcatgtacatgatcaaactggcacacatggttgatgataaacttcatgcccgttctacaggtccttactcacttgttacgcagcagcctctcggcggtaaagcccaattcggcggacagcgtttcggtgagatggaggtttgggcgcttgaagcttacggcgcagcttacacgcttcaagaaatcctgactgtgaagtccgatgacgtggtcggacgtgtgaaaacatatgaagccatcgtcaaaggcgacaatgttccagagcctggtgttccggaatcattcaaagtattgatcaaagagcttcaaagcttaggtatggacgtgaaaatcctttcaggcgatgaagaagaaatagaaatgagagatctagaagacgaggaagatgcgaaacaagctgacggccttgcattatcaggtgatgaagcgccggaagaaacagcatctccagacgttgaacgtgacgcagtaacgaaagaatag

SEQ ID NO: 3 - DNA, 1923 bp, Bacillus velezensis
  source 1..1923: mol_type = genomic DNA
atggctatggaacagcagcaaaatagttatgatgagaatcagatacaggtattagaaggtttggaagctgttcgaaagagaccggggatgtacatcggatcaactaacagcaaaggccttcaccacttggtgtgggaaatcgtcgacaacagtattgacgaagccctggccggttattgtacagatattaacatcgagattgaaaaagataacagcattaccgttaaggacaacgggcgcggaattccggtcggtatccaggagaagatgggccgccctgcggttgaagtcatcatgaccgttctccacgccggcggtaaatttgacggaagcggatataaagtatccggcggtcttcacggtgtaggggcgtctgtcgtaaacgccttgtcgaccactcttgacgttacggttcatcgtgacggaaaaatccactatcaggcgtacgagcgcggtgtacctgtggctgatcttgaagtgatcggtgatactgataagaccggaacgattacgcacttcgttccggatccggaaatcttcaaagaaacaatcgtatacgactatgatctgctttcaaaccgtgtccgggaattggccttcctgacaaaaggcgtaaacatcacgattgaagacaaacgtgaaggacaagaacggaaaaacgagtaccactacgaaggcggaatcaaaagctatgttgagtacttaaaccgttccaaagaagtcgttcatgaagagccgatttatatcgaaggcgagaaagacggcataacggttgaagttgcattgcaatacaacgacagctatacaagcaatatttattctttcacgaataatatcaacacatacgaaggcgggacgcacgaagccggatttaaaaccggtctgacccgtgtcataaacgactatgcaagaagaaaagggattttcaaagaaaatgatccgaatttaagcggggatgatgtgagagaagggctgactgccattatttcaattaagcaccctgatccgcaattcgaagggcagacgaaaaccaagctcggcaactccgaagcgagaacgatcactgatacgctgttttcttctgcgctggaaacattccttcttgaaaatccggactcagcccgcaaaatcgttgaaaaaggtttaatggccgcaagagcgcggatggcagcgaaaaaagcgcgggaattgacccggcgcaaaagtgcgcttgagatttccaatctgccgggcaaactggcggactgttcttctaaagatccgagcatttccgagctgtatatcgtagagggtgactctgcgggcggatcagcgaaacagggacgggaccgtcatttccaagctattctgccgctgcgcggtaagattctgaacgttgagaaagccagacttgataagattctctcaaacaatgaggtcagatcaatgatcacggccctcggaacaggaatcggagaagattttaatcttgaaaaagcgcgttatcataaagtggtcatcatgacggatgccgatgttgacggcgcccacatcagaacgcttttattaacgttcttctacagatacatgcgggaaatcatcgaaaacggctatgtctacattgcccagccgccgctttacaaagtgcagcagggaaaacgggtggaatacgcttataacgataagcagcttgatgagctgttaaaagagcttccgcaatcacctaagcccggcctccagcgttataaaggtcttggagaaatgaacgcgactcagctttgggaaacgacaatggaccctgcgaccagaacgcttctgcaagtcaatcttgaagatgcaatggacgctgacgagacttttgaaatgctgatgggtgacaaagtagaaccgcggagaaacttcatagaagcaaacgccagatacgtaaaaaatcttgatatttaa

SEQ ID NO: 4 - DNA, 1635 bp, Bacillus velezensis
  source 1..1635: mol_type = genomic DNA
atggcaaaagatattaagtttagtgaagaagcacgccgcgctatgcttcgcggtgtcgatgcgcttgctgacgctgtaaaagtaactttagggccaaaaggacgcaacgtggttctggagaaaaaattcggttctccgttaattacaaatgacggtgtgacaatcgcaaaagaaattgaacttgaagatgcgtttgaaaacatgggtgcgaagcttgtagctgaagtagccagcaaaacaaacgacgttgccggtgacggtacgacgactgcgactgtacttgcgcaggctatgatccgcgaaggccttaaaaacgtaactgcgggggctaaccctgtcggcgtgcgtaaaggtatggaacaagccgtgactgtagcaatcgaaaacttaaaagaaatttctaagccgatcgaaggcaaagagtctatcgctcaggttgctgcgatctctgctgctgatgaggaagtcggaagccttatcgctgaagcaatggagcgcgtaggaaacgacggcgtcatcacaatcgaagagtctaaaggattcacaactgagcttgaagttgtggaaggtatgcaattcgaccgcggatatgcgtctccttacatggtgactgactctgataagatggaagcggttctcgataatccatacatcttaatcacagacaaaaaaatcacaaacattcaagaaatccttcctgtgcttgagcaagttgtacagcaaggcaaaccattgcttctgatcgctgaagatgttgaaggtgaagctcttgctacactcgttgtcaacaaacttcgcggcacattcaacgctgttgccgttaaagctcctggcttcggtgaccgccgtaaagcaatgcttgaagacatctctgttcttactggcggagaagtaatcacagaagacttaggccttgatctgaaatctactgaaatcggacaattgggacgcgcttctaaagttgtggtaacgaaagaaaacacaacaatcgtagaaggcgccggcgacactgaaaaaatcgctgcacgcgtcaaccaaatccgcgctcaagtggaagaaacaacttctgaattcgacagagaaaaattacaagagcgtcttgcgaaacttgctggcggcgtagctgtcatcaaagtcggcgctgcgactgaaactgagctgaaagagcgtaaacttcgcatcgaagacgcactcaactccactcgcgcagctgttgaagaaggcatcgtatccggcggtggtacagcgctagtcaacgtatacaacaaagtcgctgcagtggaagctgaaggcgatgcgcaaacaggtatcaacatcgtgcttcgcgcgcttgaagagccgatccgtcaaatcgcgcacaatgctggtcttgaaggatctgtcatcgttgagcgcctgaaaaacgaaaaaatcggcgtaggcttcaacgctgcaactggcgaatgggtaaacatgatcgaaaaaggtatcgttgacccgacaaaagtgacacgttctgctctgcaaaacgcagcttctgtagcagcaatgctcttaacaactgaagccgttgtcgctgacaaaccggaagaaaacgccggcggcgcaggaatgcctgacatgggcggcatgggcggtatgggcggcatgatgtaa

SEQ ID NO: 5 - DNA, 1185 bp, Bacillus velezensis
  source 1..1185: mol_type = genomic DNA
gtgaaaaacaaatggctgtcatttttttcgggtaaagtccaaatggaagtcaaaggaaaagggattgaacggctgctgaatgaatgtacgagaaacggaatcgccatctttgcggtgaaaaaaaagcaagactgtgttctgctgatgattcagcttcaagatgtacatgctttcagaagagtcatcagaaaacatgaatgcaaagcaagctttacaaaaagaaagggtcttccctttctgcttctcaaatcaaaattaaatctgggcttcactgcgggatttgtgatattttttgttatattgtttcttttatccaacatgatttgggaaattgatattaaaggggccaagccagaaaccgagcatcagatggtaaaacaccttgaagaaatcggtgtgaaaaaaggccgtttgcagtttttaatgatgacgccggaaaaaattcaaaaatcattaacaaacggcatcgataatattacgtgggtcggtgtggaattgaacgggacagcccttcatatgaaagtggtcgaaaaaaacgaaccgacaaaagaaaagtacgtgagcccccgccatatcgttgccaaaaagaaggcggtcatcaaaaggatgttcgtgcaaaaggggcagccgatggcttttgtgaacgatcatgttgacaaaggacagctcctcgtctcaggactgatcggaaatgaagaccggaaagtcgcctcaaaagcggaaatttacggagaaacatggtacaagtcagaagtaaccgtgccccttgaaacatcatttacgctatatacgggtaaagtaaggacgaagcacaagctgtctttcggatcatggggcgtgcctttttggggcttcgggtttaatgaggagccgctgaaacatccgaaaacagaggaagaaaagcatccgtttcaatttctggggatgaagcttccggtttcttacgtttcagaacagacaagagaaagtgaaacatccgtgcggacttatacgaaaggcgaagcggttcaggccggtatcaaaatgggaagacaagatgtagaaaagcgattaaacggcagcggagaggtggaaagtgaaaaagttttgcaccaatccgttgagaatggtaaagtaaagttgattattctctaccaagttatagaagatatcgttcaaaccacacctattgttcagggagactaa

SEQ ID NO: 6 - DNA, 1773 bp, Bacillus velezensis
  source 1..1773: mol_type = genomic DNA
atgaataaacaactgaaagaaaaactggccctccttcccgatcagccgggctgttatttaatgaaagaccgccaaaaaacagtcatctacgtggggaaagcgaaagtcttgaaaaacagggtgcggtcttatttcaccggttctcacgacgcaaaaacccaacggcttgtgacggagattgaggactttgaatatatcgtgacttcctccaatcttgaagcgcttattttggaaatgaatctgattaaaaaatacgatccgaaatacaatgtcatgctgaaagatgataaaacctatccctttattaaaatcacccatgaacgccatccgcggctgattgtcacccggaatgtcaaaaaagacaaaggacgctatttcggcccgtatccgaatgtgcaggcggcgcgggaaacgaaaaaactgctggaccgcctttacccgctcaggaaatgctcaaagcttccggaccgcgtctgtctctattatcatctcggacaatgcctcgccccatgtgtaaaggatatatctgaggagacaaaccgcgagattgttgaagacatcacccgttttttaaagggagggcataacgaaatcaaaaaagagctcgaagcgaaaatggcagaagcggcggaaaagcttgaatttgaacgggctaaagaattccgcgaccagcttgctcacatcgaatcgacgatggagaagcaaaaaatgaccatgaatgaccttctggaccgcgatgtgtttgcatatgcctacgataaaggctggatgtgcgtccaagtctttttcatacgccaaggaaaactgatcgaacgcgacgtcagcatgtttccgatgtatcaggaagcggatgaagaatttctgaccttcatcggccagttctactctaaaaacaatcactttctgcctaaggaaattctggtgcctgacagcgttgacagggacatgatcaccgagctgttggaaaccgccgtgcatcagccgaaaaaaggcccgaaaaaagagctgcttttgcttgcgcacaaaaatgcgaaaatcgctctgcgggaaaaattctcgttaatcgagcgggatgaggaacggtcaatcggtgcagccgaacggctcggcgaagcgctgaatatttatacgccgcatcggattgaagcgtttgacaactccaatattcaaggcacaaaccccgtatcggccatgattgtctttattgacggaaaaccgaataaaaaggaataccgcaaatataaaattaaaaccgtaacagggccggatgattacggctcaatgagggaagtcgtcagaagaagatacacgagggtgcttcgcgaaaatcttccgctgccggatttaatcatcattgacggcggaaaagggcagattaacgcggcgcgcgacgtgctcgagaatgagctcggccttgatgtcccggtagcgggattggcgaaagatgataaacaccgaacatccaaccttttgatcggcgacccgcttgaaccggtgtttctggagcggaacagccaagagttttacctgcttcagcgcattcaggacgaagttcaccgttttgcgatcagctttcacagacagatccggggaaaaagcgtctttcaatccgttctggatgatatccccggaatcggcgaaaaacgcaaaaaaatgctcttaaaacatttcggatctgtcaaaaagatgaaggaagcaagccttgacgatatcaaaaaagcgggtgtgccggccgcggcggcccagctgctgtttgaaaaattaaaaaaatag

SEQ ID NO: 7 - DNA, 1550 bp, Bacillus velezensis; identical to SEQ ID NO: 1
  source 1..1550: mol_type = genomic DNA

SEQ ID NO: 8 - DNA, 3582 bp, Bacillus velezensis
  source 1..3582: mol_type = genomic DNA
ttgacaggtcaactagttcagtatggacgacaccgccagcgcagaagctatgctcgcattagcgaagtgttagaattaccaaatctcattgaaattcaaacctcttcttatcagtggtttcttgatgagggtcttagagagatgtttcaagacatatcaccaattgaggatttcactggtaacctctctctagagttcattgactacagtttaggagatcctaagtatcccgttgaagagtcaaaagaacgtgatgtgacttactcagctccgctgagagtgaaggttcgtttaattaacaaagaaactggagaggtaaaagaccaggatgtcttcatgggtgatttccctattatgacagataccggtacttttatcatcaacggtgcagaacgtgttatcgtatctcagcttgttcggtctccaagtgtatatttcagtggtaaagtagacaagaacggtaaaaaaggttttaccgcgactgtcattccaaaccgtggcgcatggttagaatacgaaactgatgcgaaagatgttgtgtatgtccgcattgatcgcacacgtaagttgccggttacggttcttttgcgtgctctcggcttcggttccgaccaagagattctcgatctcattggtgagaacgaatatctccgcaatacactggataaggacaacactgaaaacagtgacaaagcgcttcttgaaatctatgagcgccttcgtcccggagagccgcctacagtagaaaacgcaaaaagcttgctggattcccgtttcttcgatccgaagcgatacgaccttgcgaatgtaggacgctataaaattaataaaaagcttcatatcaagaaccgcctgtttaaccagcgccttgcagaaacactggtggatccggaaaccggtgaaattctcgctgaaaaagggcagattcttgacagaagaacacttgataaagtactgccatacttagaaaatggaatcggcttcagaaagctttatcctaacggcggcgttgtcgaggatgaagtgatgcttcaatccattaaaatctatgctcctaccgatgcagaaggagagcagacgatcaatgtgatcggcaatgcttatatcgaagaggcgattaaaaacattacgcctgctgatattatttcttctatcagctacttcttcaacctcctgcacggagtgggcgacactgatgatatcgaccatctcggaaaccgccgtctgcgttctgtaggtgagctcctgcaaaaccaattccgtatcggtttaagccggatggaacgtgtcgtacgtgaaagaatgtctattcaagacacgaatacaattacgccgcagcagctgattaacatcagacctgttattgcgtctattaaagagttcttcggaagctcacagctttctcaattcatggatcagacgaacccgcttgctgaattgacgcacaaacgccgtctgtcagctctcggaccgggcggtttgacacgtgagcgcgcaggtatggaagtacgtgacgttcactactctcactatggccgtatgtgtccgattgaaacgcctgagggcccgaacatcggtttgatcaactcattgtcatcatttgcgaaagtaaaccgctttggtttcattgagacgccataccgccgcgttgatcctgaaacaggaaaagtaacgcctagaatcgactacctgactgctgatgaagaggataactatgtcgtagcccaagcgaatgctaagctgagcgatgacggttctttcttggatgacagcatcgtagcgcgtttcagaggggaaaacaccgttgtagcccgcaaccgcgtggattacatggacgtatctcctaaacaggttgtatctgctgcgacagcatgtattccgttcttggaaaacgatgactcgaaccgcgccctcatgggagcgaacatgcagcgtcaggctgtgcctttgatgcagccggaagctccgatcgtcggaacgggtatggaatacgtatccggtaaagactccggtgcagccgttatttgtaaacaccctggtatcgttgaacgggtggaagcgaaaaacgtatgggtgcgccgctatgaagaaattgacggccaaaaagtaaaaggcaacctggataagtacagcttgctgaaatttgtccgctccaaccaaggtacgtgctacaaccagcgtccgatcgtcagtgtcggcgatgaagtagtcaaaggagaaatccttgctgacggaccttcaatggagcttggtgaacttgctctcggccgcaacgtaatggtcggcttcatgacatgggatggttacaactatgaggatgccatcatcatgagtgaacgccttgtgaaagatgatgtatacacatctattcacattgaagaatatgaatcagaagcacgtgatacaaagcttgggccggaagagatcacccgcgatattccaaacgtaggggaagacgcgcttcgcaatcttgatgaccgcggaattatccgtatcggtgcggaagtcaacgacggagaccttctcgtaggtaaagtaacgcctaaaggtgtaactgagcttacggctgaagaacgccttctgcatgcgatctttggagaaaaagcgcgtgaagtccgtgatacttctctccgtgtgcctcacggcggcggcggaattatccacgacgtaaaagtcttcaaccgtgaagacggcgacgaacttcctccgggagtgaaccagcttgtacgcgtatatatcgttcagaaacgtaagatttctgaaggtgataaaatggccggacgtcacggaaacaaaggggttatctcgaagattcttcctgaagaagatatgccttaccttcctgacggcacgccgatcgatatcatgcttaacccgctgggtgtaccatcacgtatgaatatcggtcaggtattagaacttcacatgggtatggctgcccgctacctcggcattcacatcgcgtcacctgtatttgacggcgcgcgtgaagaagatgtgtgggaaacacttgaagaagcaggcatgtcaagagacgctaaaacagttctttatgacggccgtacgggagaaccgtttgacaaccgtgtatctgtcggaatcatgtacatgatcaaactggcacacatggttgatgataaacttcatgcccgttctacaggtccttactcacttgttacgcagcagcctctcggcggtaaagcccaattcggcggacagcgtttcggtgagatggaggtttgggcgcttgaagcttacggcgcagcttacacgcttcaagaaatcctgactgtgaagtccgatgacgtggtcggacgtgtgaaaacatatgaagccatcgtcaaaggcgacaatgttccagagcctggtgttccggaatcattcaaagtattgatcaaagagcttcaaagcttaggtatggacgtaaaaatcctttcaggcgatgaagaagaaatagaaatgagagatctagaagacgaggaagatgcgaaacaagctgacggccttgcattatcaggtgatgaagcgccggaagaaacagcatctccagacgttgaacgtgacgcagtaacgaaagaatag

SEQ ID NO: 9 - DNA, 1923 bp, Bacillus velezensis
  source 1..1923: mol_type = genomic DNA
atggctatggaacagcagcaaaatagttatgatgagaatcagatacaggtattagaaggtttggaagctgttcgaaagagaccggggatgtacatcggatcaactaacagcaaaggccttcaccacttggtgtgggaaatcgtcgacaacagtattgacgaagccctggccggttattgtacagatattaacatcgagattgaaaaagataacagcattaccgttaaggacaacgggcgcggaattccggtcggtatccaggagaagatgggccgccctgcggttgaagtcatcatgaccgttctccacgccggcggtaaatttgacggaagcggatataaagtatccggcggtcttcacggtgtaggggcgtccgtcgtaaacgccttgtcgaccactcttgacgttacggttcatcgtgacggaaaaatccactatcaggcatacgagcgcggtgtacctgtggccgatcttgaagtgatcggtgatactgataagaccggaacgattacgcacttcgttccggatccggaaatcttcaaagaaacaatcgtatacgactatgatctgctttcaaaccgtgtccgggaattggccttcctgacaaaaggcgtaaacatcacgattgaagacaaacgtgaaggacaagaacggaaaaacgagtaccactacgaaggcggaatcaaaagctatgttgagtacttaaaccgttccaaagaagtcgttcatgaagagccgatttatatcgaaggcgagaaagacggcataacggttgaagttgcattgcaatacaacgacagctatacaagcaacatttattctttcacaaataatatcaacacttacgaaggcgggacgcacgaagccggatttaaaaccggtctgacccgtgtcataaacgactatgcaagaagaaaagggattttcaaagaaaatgatccgaatttaagcggggatgatgtgagagaagggctgactgccattatttcaattaagcaccctgatccgcaattcgaagggcagacgaaaaccaagctcggcaactccgaagcgagaacgatcactgatacgctgttttcttctgcgctggaaacattccttcttgaaaatccggactcagcccgcaaaatcgttgaaaaaggtttaatggccgcaagagcgcggatggcagcgaaaaaagcacgggaattgacccggcgcaaaagtgcgcttgagatttccaatctgccgggcaaactggcggactgttcttctaaagatccgagcatttccgagctgtatatcgtagagggtgactctgcgggcggatcagcgaaacagggacgggaccgtcatttccaagctattctgccgctgcgcggtaagattctgaacgttgagaaagccagacttgataagattctctcaaacaatgaggtcagatcaatgatcacggccctcggaacaggaatcggagaagattttaatcttgaaaaagcgcgttatcataaagtggtcatcatgacggatgccgatgttgacggcgcccacatcagaacgcttttattaacgttcttctacagatacatgcgggaaatcatcgaaaacggctatgtctacattgcccagccgccgctttataaagtgcagcagggaaaacgggtggaatacgcttataacgataagcagcttgatgagctgttaaaagaacttccgcaatcacctaagcccggcctccagcgttataaaggtcttggagaaatgaacgcgactcagctttgggaaacgacaatggaccctgcgaccagaacgcttctgcaagtcaatcttgaagatgcaatggacgctgacgagacttttgaaatgctgatgggtgacaaagtagaaccgcggagaaacttcatagaagcaaacgccagatacgtgaaaaatcttgatatttaa

SEQ ID NO: 10 - DNA, 1635 bp, Bacillus velezensis
  source 1..1635: mol_type = genomic DNA
atggcaaaagatattaagtttagtgaagaagcacgccgcgctatgcttcgcggtgtcgatgcgcttgctgacgctgtaaaagtaactttagggccaaaaggacgcaacgtggttctggagaaaaaattcggttctccgttaattacaaatgacggtgtgacaatcgcaaaagaaattgaacttgaagatgcgtttgaaaacatgggtgcgaagcttgtagctgaagtagccagcaaaacaaacgacgttgccggtgacggtacgacgactgcgactgtacttgcgcaggctatgatccgcgaaggccttaaaaacgtaactgcgggggctaaccctgtcggcgtgcgtaaaggtatggaacaagccgtgactgtagcaatcgaaaacttaaaagaaatttctaagccgatcgaaggcaaagagtctatcgctcaggttgctgcgatctctgctgctgatgaggaagtcggaagccttatcgctgaggcaatggagcgcgtaggaaacgacggcgtcatcacaatcgaagagtctaaaggattcacaactgagcttgaagttgtggaaggtatgcaattcgaccgcggatatgcgtctccttacatggtgactgactctgataagatggaagcggttctcgataatccatacatcttaatcacagacaaaaaaatcacaaacattcaagaaatccttcctatgcttgagcaagttgtacagcaaggcaaaccattgcttctgatcgctgaagatgttgaaggtgaagctcttgctacactcgttgtcaacaaacttcgcggcacattcaacgctgttgccgttaaagctcctggcttcggtgaccgccgtaaagcaatgcttgaagacatctctgttcttactggcggagaagtaatcacagaagacttaggccttgatctgaaatctactgaaatcggacaattgggacgcgcttctaaagttgtggtaacgaaagaaaacacaacaatcgtagaaggcgccggcgacactgaaaaaatcgctgcacgcgtcaaccaaatccgcgctcaagtggaagaaacaacttctgaattcgacagagaaaaattacaagagcgtcttgcgaaacttgctggcggcgtagctgtcatcaaagtcggcgctgcgactgaaactgagctgaaagagcgtaaacttcgcatcgaagacgccctcaactcaactcgcgcagctgttgaagaaggtatcgtatccggcggtggtacagcgcttgtcaacgtatacaacaaagtcgctgcagtggaagctgaaggcgatgcgcaaacaggtatcaacatcgtgcttcgcgcgcttgaagagccgatccgtcaaatcgcgcacaatgctggtcttgaaggatctgtcatcgttgagcgcctgaaaaacgaaaaaatcggcgtaggcttcaacgctgcaactggcgaatgggtaaacatgatcgaaaaaggtatcgttgacccgacaaaagtgacgcgttctgctctgcaaaacgcagcttctgtagcagcaatgctcttaacaactgaagccgttgtcgctgacaaaccggaagaaaacgccggcggcgcaggaatgcctgacatgggcggcatgggcggtatgggcggcatgatgtaa

SEQ ID NO: 11 - DNA, 1131 bp, Bacillus velezensis
  source 1..1131: mol_type = genomic DNA
atggcatcagtaaaaaaagataaaagaaacggcaattggtactatgtgtttgatataggaaaagatgagaacggcagacggaagcaacgtaaacgaagtgggttcaagctaaaaaaagatgcagaagaagcattaagggaagatcttcagttataccatgctggggatcttctcaaagataatgattcaactttcaaagaattggttgagtattggctgaatatcaaaactccagatgtgagcaaccaaactctaaaggtttatcattataatctaaaaaatcatatactccctaccttcggaagcatgaaacttagcgatataacaactcaaaaggtacaagcatttataacaaggttagttaattccggtttatcggctgccacaataaagaagatatatcacgtactcaacaacgtaatgaaaacagctgttcaagatgagtttattaaaaagaatccagttgaaaaggttagaaagccatcagttaagcgtaaagaagttgaagtatggtcagccgaacagatgtcattattcctggatcacaccaaaaacagtcgttactatattgcattttggttagcgatttctttcggacttagacaaggtgaaattttaggtttacgttttaaggatatagacttcaataatggcgttttgagaatcgttcaaacactagaacattctggcggccaaacaaaatacggtggaaaatcatcgacaagcacacgcaccatcgacttatcagaacatgatatccatatactgaagaaacaaagaagtcgtgtattgaaagagaagagtttatgcggagggctctatacagaccgagatttagttgtatgtacagatacagggaatgcaatcaatccaagaaaccttttaagacagttcaaagcttatttaaagcagcttgatttacctgatatcccattccataaccttagacactctcatgcatccttactgttaacaaagtttcatcctaaagttgttcaagaaaggttaggacataaagatatccaggtcacgcttaacacctattcgcatttaatgccaaacatgcagaaggatgcttccacatttatcagtggcatcttacaaggcaaacaaaaagaggaatcacattaa

SEQ ID NO: 12 - DNA, 1077 bp, Bacillus velezensis
  source 1..1077: mol_type = genomic DNA
ttggctgattatatagaagtaaaagcatttttctttggaaatgaggccgaaaaagaacaagtatatcttaattttattttaccgtttttttccccgatccttggtcgttttcatgcagagcggggatggaccggaggaccgcactttcgaattatattgtcaaaaagtgatacaagtataattgaaacatttccaagtgaatttaagcgatactgcacaacacattttcctgaattaacacaggtcgagatagaaaacaatttgtccccttatttgactcatcaagatattataccgaatatggaaagaagagaaagcattccaattttgattgagaatcatttaagcgttctaatcggaccctacaatgaagaatatatgtataacacttttaattcttacgctcattttgtagcgcataccagagccctttttatgatgcaagagtttatttctgttaatatttataaattcaaagaaataagcccagaaacacagctcaaaactttgacaagaatgctttatgatgttttagcattttccagttatacggacaaattctctgtgctagtttatgtttcaaatacggaaggcgttttttcaatagctgatagtctaaataaaaaaaggtcatttgaagactcattcttaaaaatgtacaaagctttagaaatccctgcctattttacaaatcaatcatacaatctatctatcggttcaagctggtttgatactgtttcaaaaatcgtagattatacaaaaaaaaatttagatgctttagcagattcagaagatggattttattcgattgaaaaacagaaagaagatttagtaaagaatattgaaagtattgatagcccttttcataagaatctcttaaatcaaattgattcattacttaatcataatgagcataaaatgttcaagtttttaatcaatatcatttataagtcagttcatatgttggggtttacttttgttaagaaaaattttgcttgctttgctgtttccaaatatgtattagataagcatcatacaacatgggaagagattttaaaagaaagagagcgagtataa

SEQ ID NO: 13 - DNA, 1550 bp, Bacillus subtilis
  source 1..1550: mol_type = genomic DNA
ttatcggagagtttgatcctggctcaggacgaacgctggcggcgtgcctaatacatgcaagtcgagcggacagatgggagcttgctccctgatgttagcggcggacgggtgagtaacacgtgggtaacctgcctgtaagactgggataactccgggaaaccggggctaataccggatggttgtttgaaccgcatggttcaaacataaaaggtggcttcggctaccacttacagatggacccgcggcgcattagctagttggtgaggtaacggctcaccaaggcaacgatgcgtagccgacctgagagggtgatcggccacactgggactgagacacggcccagactcctacgggaggcagcagtagggaatcttccgcaatggacgaaagtctgacggagcaacgccgcgtgagtgatgaaggttttcggatcgtaaagctctgttgttagggaagaacaagtaccgttcgaatagggcggtaccttgacggtacctaaccagaaagccacggctaactacgtgccagcagccgcggtaatacgtaggtggcaagcgttgtccggaattattgggcgtaaagggctcgcaggcggtttcttaagtctgatgtgaaagcccccggctcaaccggggagggtcattggaaactggggaacttgagtgcagaagaggagagtggaattccacgtgtagcggtgaaatgcgtagagatgtggaggaacaccagtggcgaaggcgactctctggtctgtaactgacgctgaggagcgaaagcgtggggagcgaacaggattagataccctggtagtccacgccgtaaacgatgagtgctaagtgttagggggtttccgccccttagtgctgcagctaacgcattaagcactccgcctggggagtacggtcgcaagactgaaactcaaaggaattgacgggggcccgcacaagcggtggagcatgtggtttaattcgaagcaacgcgaagaaccttaccaggtcttgacatcctctgacaatcctagagataggacgtccccttcgggggcagagtgacaggtggtgcatggttgtcgtcagctcgtgtcgtgagatgttgggttaagtcccgcaacgagcgcaacccttgatcttagttgccagcattcagttgggcactctaaggtgactgccggtgacaaaccggaggaaggtggggatgacgtcaaatcatcatgccccttatgacctgggctacacacgtgctacaatggacagaacaaagggcagcgaaaccgcgaggttaagccaatcccacaaatctgttctcagttcggatcgcagtctgcaactcgactgcgtgaagctggaatcgctagtaatcgcggatcagcatgccgcggtgaatacgttcccgggccttgtacacaccgcccgtcacaccacgagagtttgtaacacccgaagtcggtgaggtaaccttttaggagccagccgccgaaggtgggacagatgattggggtgaagtcgtaacaaggtagccgtatcggaaggtgcggctggatcacctccttt

SEQ ID NO: 14 - DNA, 3582 bp, Bacillus subtilis
  source 1..3582: mol_type = genomic DNA
ttgacaggtcaactagttcagtatggacgacaccgccagcgcagaagctatgctcgcattagcgaagtgttagaattaccaaatctcattgaaattcaaacctcttcttatcagtggtttcttgatgagggtcttagagagatgtttcaagacatatcaccaattgaggatttcactggtaacctctctcttgagttcattgattatagtttaggtgagcctaaatatcctgtagaggaatcaaaagaacgtgatgtgacttactcagctccgctaagagtgaaggttcgtttaattaacaaagaaactggagaggtaaaagaccaagatgtcttcatgggtgatttccctattatgacagatacaggtacttttatcattaacggtgcggaacgtgttattgtttcccagcttgttcggtctccaagtgtatatttcagtggtaaagtagacaaaaacggtaaaaaaggttttaccgcaactgtcattccaaaccgtggcgcatggttagaatacgaaactgatgcgaaagatgttgtttatgtccgcattgatcgcacacgtaagttgccggttacggttcttttgcgtgctctcggcttcggctccgatcaagagattcttgatctcataggagaaaacgaatacctgcgaaatacgcttgataaagataacacagaaaacagtgacaaagcgttgctggaaatttacgagcgtctccgtcctggagagccgcctacagtagaaaatgcgaaaagcttgcttgattctcgtttctttgatccgaaacgatacgatcttgccaatgtaggacgctataaaattaataaaaaacttcatattaagaatcgcctcttcaatcagagacttgctgaaacgcttgttgatcctgaaacaggagaaatccttgctgaaaaaggccagattcttgatagaagaacacttgataaagtactgccatacttagaaaacggaatcggttttagaaagctgtatccgaatggcggcgttgttgaagatgaagtgactcttcaatcaattaaaatctttgctccgactgatcaagaaggagaacaggttattaatgtaatcggcaatgcttacatcgaagaagagattaaaaacatcacgcctgctgatattatttcttcaatcagctacttcttcaacttgctgcacggagtaggcgatacagatgatatcgatcatcttggaaaccgccgtttacgctctgtaggcgagcttctccagaaccaattccgtatcggtttaagccgtatggaacgtgtggttcgtgagagaatgtcaattcaagatacgaatacaattacgcctcagcagctgatcaatattcgtcctgttattgcgtccattaaagagttctttggaagctcacagctttctcaattcatggatcagacgaacccgcttgctgaattaacgcacaagcgtcgtctgtcagcattaggaccgggcggattgacacgtgagcgtgccggaatggaagtgcgtgacgttcactactcccactatggccgtatgtgtccgattgaaacgcctgagggcccgaacatcggtttgatcaactcactatcatcttatgcaaaagtaaaccgttttggctttattgaaacgccatatcgccgcgttgaccctgaaacagggaaggtaacgggcagaatcgattacttaactgctgatgaagaggataactatgttgtcgctcaagcgaatgctcgtcttgatgacgaaggcgcctttattgatgacagcatcgtagctcgtttccgcggggagaacactgttgtttccagaaaccgtgtagactacatggatgtatcgcctaagcaggttgtatctgctgcgacagcatgtatcccgttcttagaaaacgatgactcgaaccgtgccctcatgggagcgaacatgcagcgccaggctgtgcctttgatgcagccggaagctccatttgttggaactggtatggaatacgtatcaggaaaagactctggtgccgctgttatttgtaaacaccctggtatcgttgaacgcgtagaagcgaaaaacgtttgggttcgccgttatgaagaagtagacggtcaaaaagtaaaaggaaacctggataaatacagcctgctgaaatttgtccgctctaaccaaggtacgtgctacaaccagcgtccgatcgtaagtgtcggcgatgaagtggtaaaaggagaaatccttgctgacggtccttctatggagcttggtgaacttgcacttggccgtaacgtaatggtcggcttcatgacatgggatggctacaactatgaggatgccatcatcatgagtgaacgcctagtgaaggatgatgtttatacatctatccacattgaagaatacgaatcagaagcacgtgatacgaaacttggacctgaagaaatcactcgcgatattccaaacgtcggtgaagatgcgcttcgcaatcttgatgaccgtggaatcatccgtattggggcagaagtaaaagacggagatcttcttgttggtaaagtaacgcctaaaggcgtaactgaactgactgcagaagaacgccttcttcacgccatttttggcgagaaagcccgcgaggttcgtgatacttctcttcgtgtgcctcacggcggcggcggaattatccatgacgttaaagtcttcaaccgtgaagacggagacgaacttcctccaggtgttaaccagttagtacgcgtatatatcgttcagaaacgtaagatttctgaaggggataaaatggccggtcgtcacggtaacaaaggtgttatctctaagattcttcctgaagaggatatgccttaccttcctgacggcacaccaattgatatcatgcttaacccgctgggcgtaccatcacgtatgaacatcgggcaggtattggaacttcacatgggtatggccgctcgttaccttggcattcacattgcatctcctgtatttgacggagcgcgagaagaggatgtctgggaaacacttgaagaagccggcatgtctcgtgacgccaaaacagtgctttacgacggacgtactggagagccgtttgataaccgtgtatctgtcggtatcatgtacatgatcaaactagctcacatggttgacgataaacttcatgcacgctctacaggtccttactcacttgttacgcagcagcctcttggcggtaaagcgcaatttggcggacagcgttttggtgagatggaggtttgggcacttgaagcttacggtgcggcttatactcttcaagaaattctgactgttaagtctgatgacgtggttggacgtgtgaaaacatacgaagccatcgttaaaggcgacaatgttcctgaaccaggtgttccggaatcattcaaagtattaatcaaagaacttcaaagcttaggtatggatgtcaaaatcctttctggtgatgaagaagaaatagaaatgagagatttagaagacgaagaagatgcgaaacaagctgacggcctggcattatcaggtgatgaagagccggaagaaacagcatctgcagacgttgaacgcgatgtagtaacaaaagaataa

SEQ ID NO: 15 - DNA, 1923 bp, Bacillus subtilis
  source 1..1923: mol_type = genomic DNA
gtggctatggaacagcagcaaaacagttatgatgaaaatcagatacaggtactagaaggattggaagctgttcgtaaaagaccggggatgtatatcggttcgacaaacagcaaaggccttcaccacctggtatgggaaattgtcgacaatagtattgacgaagccctcgccggttattgtacggatatcaatatccaaatcgaaaaagacaacagtatcacggttgtagataatggccgcggtattccagtcggtattcatgaaaaaatgggccgtcctgcggtagaagtcattatgacggtacttcatgccggaggaaaatttgacggaagcggctataaagtatccggaggattacacggtgtaggtgcgtctgtcgtaaacgcactatcaacagagcttgatgtgacggttcaccgtgacggtaaaattcaccgccaaacttataaacgcggagttccggttacagaccttgaaatcattggcgaaacggatcatacaggaacgacgacacattttgtcccggaccctgaaattttctcagaaacaaccgagtatgattatgatctgcttgccaaccgcgtacgtgaattagcctttttaacaaagggcgtaaacatcacgattgaggataaacgtgaaggacaagagcgcaaaaatgaataccattacgaaggcggaattaaaagttatgtagagtatttaaaccgctctaaagaggttgtccatgaagagccgatttacattgaaggcgaaaaggacggcattacggttgaagtggctttgcaatacaatgacagctacacaagcaacatttactcgtttacaaacaacattaacacgtacgaaggcggtacccatgaagctggcttcaaaacgggcctgactcgtgttatcaacgattacgccagaaaaaaagggcttattaaagaaaatgatccaaacctaagcggagatgacgtaagggaagggctgacagcgattatttcaatcaaacaccctgatccgcagtttgagggccaaacgaaaacaaagctgggcaactcagaagcacggacgatcaccgatacgttattttctacggcgatggaaacatttatgctggaaaatccagatgcagccaaaaaaattgtcgataaaggcttaatggcggcaagagcaagaatggctgcgaaaaaagcccgtgaactaacacgtcgtaagagtgctttggaaatttcaaacctgcccggtaagttagcggactgctcttcaaaagatccgagcatctccgagttatatatcgtagagggtgactctgccggaggatctgctaaacaaggacgcgacagacatttccaagccattttgccgcttagaggtaaaatcctaaacgttgaaaaggccagactggataaaatcctttctaacaacgaagttcgctctatgatcacagcgctcggcacaggtattggggaagacttcaaccttgagaaagcccgttaccacaaagttgtcattatgacagatgccgatgttgacggcgcgcacatcagaacactgctgttaacgttcttttacagatatatgcgccaaattatcgagaatggctacgtgtacattgcgcagccgccgctctacaaggttcaacaggggaaacgcgttgaatatgcgtacaatgacaaggagcttgaagagctgttaaaaactcttcctcaaacccctaagcctggactgcagcgttacaaaggtcttggtgaaatgaatgccacccagctatgggagacaaccatggatcctagctccagaacacttcttcaggtaactcttgaagatgcaatggatgcggacgagacttttgaaatgcttatgggcgacaaggtagaaccgcgccgaaacttcatagaagcgaatgcgagatacgttaaaaatcttgacatctaa

SEQ ID NO: 16 - DNA, 1632 bp, Bacillus subtilis
  source 1..1632: mol_type = genomic DNA
atggcaaaagaaattaagtttagtgaagaagctcgccgcgcaatgcttcgcggtgtcgatgcacttgctgatgctgttaaagtaactttaggaccaaaaggacgcaacgtggttctagagaaaaaattcggttctccgttaatcacaaatgacggtgtaacaatcgctaaagaaatcgagctagaagacgcttttgaaaacatgggtgctaagcttgttgctgaagtagccagcaaaacaaacgacgttgccggtgacggtacaacaactgcaacagttcttgcgcaagcaatgatccgtgaaggccttaaaaacgtaacagcaggcgctaaccctgtaggcgtgcgtaaagggatggaacaagctgtagcggttgcgatcgaaaacttaaaagaaatttctaagccaatcgaaggcaaagagtctatcgctcaggttgctgcgatctctgctgctgacgaggaagtcggaagccttatcgctgaagcaatggagcgcgtaggaaacgacggcgttatcacaatcgaagagtctaaaggcttcacaactgagcttgaagttgttgaaggtatgcaattcgaccgcggatatgcgtctccttacatggtaactgactctgataagatggaagcggttcttgacaatccttacatcttaatcacagacaaaaaaatcacaaacattcaagaaatccttcctgtgcttgagcaggttgttcagcaaggcaaaccattgcttctgatcgctgaggatgttgaaggcgaagcacttgcaacacttgttgtgaacaaacttcgcggcacattcaacgcagttgctgttaaagctcctggcttcggtgaccgccgtaaagcaatgcttgaagacatcgctgtccttactggcggagaagtcatcacagaagatcttggccttgacctgaaatctactcaaatcgctcaattgggacgcgcttctaaagttgtcgttactaaagaaaacacaacaatcgttgaaggcgctggcgaaacagacaaaatttctgcccgcgtgactcaaatccgcgctcaagtggaagaaacaacttctgagttcgacagagaaaaattacaagagcgtcttgcgaaacttgctggcggcgtagctgtcatcaaagtcggcgctgcgactgaaactgagctgaaagagcgtaaacttcgcatcgaagacgccttgaactcaactcgcgcagctgttgaagaaggcatcgtatccggtggtggtacagcgcttgtaaacgtatataacaaagtcgctgcagttgaagctgaaggcgatgctcaaacaggtatcaacatcgtgcttcgcgcgcttgaagagccaatccgtcaaatcgcacacaacgctggccttgaaggatctgtcatcgttgagcgcctcaaaaacgaagaaatcggcgtaggcttcaacgctgcaactggcgaatgggtaaacatgatcgaaaaaggtatcgttgacccaacgaaagttacacgctcagctcttcaaaacgctgcgtctgtagctgcaatgttcttaactactgaagctgttgtcgctgacaagccagaagaaaacgctggcggcggaatgcctgacatgggcggcatgggcggtatgggcggcatgatgtaa

SEQ ID NO: 17 - DNA, 642 bp, Bacillus subtilis
  source 1..642: mol_type = genomic DNA
atggtgcttcgatatacagctctgggcgattccttgacgacagggagaggctccgggctgttttcacccggcttcgtccagcgttttggggacatgatggaagctgacttgaaaacaagaacggcaataaacatatttgccagatcaggcctgaatacagaagagattttgggactcctgtcatatccctatgtgcaaaaatgtattcgagatgctgatatgataacgatcacagggtgcggaaacgatctcatcgattcggtcttagcctaccaaacctctaaggatgaaacgattttcagccgtgtatccgcccattgccatgagaattttgaaaagatgattgccaaagtcgccgagattaaaggagaaaatccttccccgtacgccattcgtgtgttcaacttatacaatccgtttcccgaaattgatatcgccggcaaatggatcacttcgtttaattcacatttagaaacacttgcatcagcaccccatgtcaaaatcgcggatgcctatagcatcttcaaaggcaaagaacaggaatatctgtcctttgacggtgtccatccgaacagcaaaggctatcaagcgatggctgaagccgttcacaagctaggctataaagaattatcagtttcatag

SEQ ID NO: 18 - DNA, 579 bp, Bacillus subtilis
  source 1..579: mol_type = genomic DNA
ttgagcaaactcgatgaaatgactgcttacctgccgccgttccttaccaaattgaaagaaatggcggaacttcttcaggcagaagctccggaatttgaaaagcaaaataatagcatctttgatctgacagatcagttgtttgttactacggcaacctgggggcttgaacgatgggaaaagattttgaacgtaccgcgggaatcaggtgaccccgatgagatccgccgattgcgtctaatctctaaaatgtccaatataccgccggcaacatataaggccattgaacaggcattgaaccggttcctgaaaaatccgtctgctcaggtcaggctgcttcaaggacagtaccgttttaatgttgatattgatatagatgatatgcagcatatgagcgagctcatagaaacattggagaatatgaagccagctcatttggcatataccttgcgagctgctgtgaatgagccactcaagataaaagatactgtcattttgaataacagaaggtatcgaaaagcaagtgagctaaaggtaggttattccgtcacgctcaataataacgaggtggtccttgcatga

SEQ ID NO: 19 - DNA, 1550 bp, Bacillus licheniformis
  source 1..1550: mol_type = genomic DNA
ttcatggagagtttgatcctggctcaggacgaacgctggcggcgtgcctaatacatgcaagtcgagcggaccgacgggagcttgctcccttaggtcagcggcggacgggtgagtaacacgtgggtaacctgcctgtaagactgggataactccgggaaaccggggctaataccggatgcttgattgaaccgcatggttcaatcataaaaggtggcttttagctaccacttacagatggacccgcggcgcattagctagttggtgaggtaacggctcaccaaggcgacgatgcgtagccgacctgagagggtgatcggccacactgggactgagacacggcccagactcctacgggaggcagcagtagggaatcttccgcaatggacgaaagtctgacggagcaacgccgcgtgagtgatgaaggttttcggatcgtaaaactctgttgttagggaagaacaagtaccgttcgaatagggcggtaccttgacggtacctaaccagaaagccacggctaactacgtgccagcagccgcggtaatacgtaggtggcaagcgttgtccggaattattgggcgtaaagcgcgcgcaggcggtttcttaagtctgatgtgaaagcccccggctcaaccggggagggtcattggaaactggggaacttgagtgcagaagaggagagtggaattccacgtgtagcggtgaaatgcgtagagatgtggaggaacaccagtggcgaaggcgactctctggtctgtaactgacgctgaggcgcgaaagcgtggggagcgaacaggattagataccctggtagtccacgccgtaaacgatgagtgctaagtgttagagggtttccgccctttagtgctgcagcaaacgcattaagcactccgcctggggagtacggtcgcaagactgaaactcaaaggaattgacgggggcccgcacaagcggtggagcatgtggtttaattcgaagcaacgcgaagaaccttaccaggtcttgacatcctctgacaaccctagagatagggcttccccttcgggggcagagtgacaggtggtgcatggttgtcgtcagctcgtgtcgtgagatgttgggttaagtcccgcaacgagcgcaacccttgatcttagttgccagcattcagttgggcactctaaggtgactgccggtgacaaaccggaggaaggtggggatgacgtcaaatcatcatgccccttatgacctgggctacacacgtgctacaatgggcagaacaaagggcagcgaagccgcgaggctaagccaatcccacaaatctgttctcagttcggatcgcagtctgcaactcgactgcgtgaagctggaatcgctagtaatcgcggatcagcatgccgcggtgaatacgttcccgggccttgtacacaccgcccgtcacaccacgagagtttgtaacacccgaagtcggtgaggtaaccttttggagccagccgccgaaggtgggacagatgattggggtgaagtcgtaacaaggtagccgtatcggaaggtgcggctggatcacctccttt

SEQ ID NO: 20 - DNA, 3582 bp, Bacillus licheniformis
  source 1..3582: mol_type = genomic DNA
ttgacaggtcaactagttcagtatggacgacaccgccagcgcagaagctatgcacgcattagcgaagtgttagaattaccaaatctcattgaaattcaaacctcttcttatcagtggtttcttgatgagggtcttagagagatgtttcaagacatatcgccaattgaggatttcactggtaacctctctctggaatttatcgactacagcttgggcgagcctaagtatccggtagaagaatcaaaagagcgggatgtgacctattcagctccgctgcgggttaaagtccgcttaatcaacaaagaaaccggcgaagtaaaggatcaggatgtcttcatgggcgatttccctattatgacagacactggaaccttcattatcaacggtgcagaacgggtcatcgtatctcagctcgttcgttctccaagtgtatattttagtggtaaagtagacaaaaacggtaagaaaggttttaccgcgactgtcattccaaaccgtggcgcatggttagaatacgagactgatgcgaaagatgttgtttacgtacgcatcgatcgcacacgtaagttgccggttacggttcttttgcgtgctcttggcttcggatctgaccaagagatcattgatctcatcggtgaaaacgagtatctgcgcaatacgcttgataaagataatacggaaaacaccgataaagcgcttcttgaaatctacgagcgtcttcgtccaggggagccgcctaccgtagaaaacgcaaaaagcctgcttgattcaaggttctttgatccgaaaagatatgaccttgcgagtgtaggacgttataaaattaataaaaagcttcacatcaaaaaccgactttttaatcagcggcttgctgaaacgctagtcgaccctgaaacaggcgaaatccttgccgaaaaaggagcgattttagacagaagaacgcttgataaagttctgccgtaccttgaaaacggaatcggttttaaaaagctttatccgaacggcggagttgtcgaagacgaagtaacgcttcagtctatcaaaatctatgctccgacagaccaagaaggggagcagacaatcaatgtgattggaaatgcttatatcgaagaaggcgttaagaatattacaccttctgatattatcgcttccatcagctatttctttaacctgcttcacggagtgggcgataccgacgatatcgaccatctaggaaaccgccgtctccgttcagtgggagagcttctgcaaaaccaattccgtattggtttaagcagaatggagcgcgttgttcgtgaaagaatgtctattcaagatacaaacacgatcacgccgcagcagctgatcaatattcgccctgtcatcgcatcaatcaaagagtttttcggaagctcgcagctttctcagtttatggatcagacgaatccgcttgctgagctgacgcataagcgccgtctgtcagcgctcggaccgggcggtttgactcgtgagcgcgccggaatggaagtccgtgacgttcactattcacactacggccggatgtgtccgattgaaacccctgagggtccaaacatcggcttgatcaactcgctttcttcattcgcgaaagtgaaccgtttcggcttcatcgaaacgccgtatcgccgcgtcgatcctgaaactggaaaagtaacgccgagaatcgattacttgacagctgatgaagaagacaactatgtcgttgcccaggcaaacgcacgcctgaatgatgacggttcttttgtggatgacagcatcgtcgcccgtttcagaggggagaacaccgttgttccgaaagaccgcgtcgactatatggacgtttcgcctaaacaggttgtctctgccgcgactgcatgtattcctttcttggaaaacgatgactcaaaccgcgcccttatgggagcgaacatgcaacgtcaggccgtacctcttatgcagcctgaatcgccgatcgtcggaaccgggatggaatatgtatctgcgaaagactccggtgccgctgttatttgccgccaccctggaatcgttgaacgggtggaagcgaagaacatctgggtgcgccgctatgaagaagtcgacggccagaaagtcaaagggaaccttgataaatacagcctgctgaagtttgtccgttccaaccagggaacttgctacaaccagcgtccgatcgtaagcgtcggtgatgaggttgaaaaaggtgaaattttagctgacggtccgtccatggaaaaaggtgagcttgcccttggacgcaacgtcatggtcggctttatgacatgggatggctacaactatgaggatgccatcatcatgagcgaacgccttgtaaaagacgacgtatacacgtctattcatattgaagaatacgaatcagaggcccgggatacaaaactcggacctgaagaaatcactcgcgatattccgaacgtcggtgaggacgctcttcgcaatctcgatgaacgcggaattatccgtgtcggtgctgaagtaaaagacggagatcttcttgttggtaaagtaacccctaaaggtgttacagagcttacggcggaagaacgcctgcttcatgccatcttcggggaaaaagcgcgtgaagtgcgtgatacgtcgctgcgtgtacctcacggaggcggcggtatcatccttgatgtaaaagtgttcaaccgcgaagacggagacgaactgcctccgggcgttaaccagctcgtccgcgtctacatcgttcagaagcgtaaaatttctgaaggggacaaaatggccggacgccacggtaacaaaggtgttatttcgaaaattcttccggaggaagatatgccgtatctgcctgacggaacgccgattgacatcatgttaaacccgctgggcgtaccatcgcgtatgaacatcgggcaggtgttggagctgcaccttggtatggctgcacgccgcctcggtctgcatgtcgcgtcacctgtatttgacggtgcccgcgaagaagatgtgtgggaaacccttgaagaagccggcatgtcaagagacgcaaaaaccgtcctttacgacggccgaactggggagccgtttgacaaccgggtttctgtcggcatcatgtacatgatcaaactggcacacatggttgacgacaaattgcacgcacgttcaaccggtccttactcactcgttacccagcagcctctcggaggtaaagcgcagttcggcggacagcgttttggagagatggaagtttgggcgcttgaagcttatggtgcagcatatacgctacaagagatcctgactgttaaatcggatgatgtcgtaggccgtgtgaaaacatatgaagccatcgtaaaaggcgacaatgttccagaacctggtgttccggaatcgttcaaagtattgatcaaagagcttcaaagcttaggtatggacgtcaaaattctatcaagcgacgaagaagaaatcgaaatgagagacttggaagacgacgaagacgcgaaacaaaacgaagggctttctctgccgaatgatgaagagtccgaagagttggtttctgctgacgcagaacgcgatgtcgttacaaaagaataa

SEQ ID NO: 21 - DNA, 1920 bp, Bacillus licheniformis
  source 1..1920: mol_type = genomic DNA
gtggcaatggaacagcaaaataattacgatgaaaatcagatacaggttctagagggattggaagccgttcggaaaagacccggaatgtacatcgggtcgacaagcggcaaaggtctgcaccatttagtatgggaaattgtcgataacagcatcgatgaagcattggccggttactgcactgaaatcaatgtcgcaattgaaaaagacaacagcatcacagtaaaagacaacggacggggtatcccggtcggtattcatgagaagatgggtcgtcccgctgtggaagtcatcatgactgtcctgcacgccggaggaaagtttgacggaagcggatataaagtttcgggcggtttgcacggcgtcggtgcttctgttgttaacgccctttcaaccgagctggatgtaacggtttacagagatggaaaaatccattatcaggaatttgaacgtggcgttccgaaagctgatttgaaagtcattggagatacggaagtgacgggaacgaccacacacttcaagcctgatccggaaatattcacggaaacgactgaatacgactatgatacgctcgccactcgtgtccgcgaactcgctttcttgacaaaaggcgtcaaaatcacgatcgaagacaagcgagaaggaaaagaacgcaagaatgaatactgctatgaaggcggtattaaaagctatgttgaacacttgaaccgttcgcgggaagttattcatgaagagccggtctatattgaaggatccaaagacggcattacagtcgaggtggctcttcaatacaatgacagctatacaagcaacatttattcatttgctaacaacattcatacgtatgaaggcggaacccatgaagccggctttaagaccggtttgacgagggtcatcaatgattacgcgagaagaaacggcgtattcaaagaaagcgatccgaacttaagcggagaagacgtccgggaaggtttgacagcgattatttcaatcaagcacccggatcctcaatttgaagggcagacgaaaacaaagctcggcaactcagaagcgcgtacgataacagatgcgctattttcagaagcgcttgaaaagtttctgctagaaaacccggattcagcgaaaaaaatcgttgaaaaaggggttatggccgccagagcacggatggctgcaaagaaagcacgcgaattgacgcgcagaaaaagcgcccttgaagtgtccaatctgccggggaaacttgctgactgttcttctaaagacccgacgatttccgaactttacatcgttgagggtgactctgcgggcggatcggcaaaacagggccgcgaccgtcatttccaagcaattttgcctttgagagggaaaattttgaacgtcgaaaaagcccgcctggacaaaatattgtccaacaatgaggttcgttctatgatcaccgcccttggcaccggaatcggggaagatttcaaccttgaaaaagcccgctaccacaaagtcgtgattatgacggatgccgacgtcgatggtgcacacatcagaacattgctgctgacctttttctaccgctacatgagacagattatcgaacaaggatatgtctacatcgctcagccgcctctttacaaagtacagcaggggaaacgcgttgagtatgcgtacaatgaccagcagctcgaagaaattttaaaagagcttccgcaaaatcctaagccaggcctgcagcgctacaaaggtttgggcgagatgaatgcgacacagctttgggaaacgacgatggatccagaaacgcggacattgcttcaagtaacgctcaaagatgcgattgatgcggatgaaacctttgaaatgctgatgggcgacaaggttgaaccgcgccgcaacttcatcgaagagaatgcccgatatgtaaagaatttggatatttaa

SEQ ID NO: 22 - DNA, 1635 bp, Bacillus licheniformis
  source 1..1635: mol_type = genomic DNA
atggcaaaagatattaagtttagcgaagaagcccgccgttcaatgctgcgcggtgtagatgcattggcggatgctgtaaaggtaactttgggacctaaaggacgcaacgtcgttcttgagaaaaaattcggttctccattaatcacaaacgacggtgtaaccatcgcgaaagaaatcgagcttgaagacgcgttcgaaaacatgggcgcaaagcttgttgctgaagttgcgagcaaaacaaacgatgttgccggtgacggtacaacaacagcgacagttctagctcaggcgatgattcgcgaaggtcttaaaaacgtaactgccggcgctaaccctgtaggcgtgcgcaaaggtatcgagcaggctgtggctgtagctgttgaaagcctgaaagaaatctctaaaccaatcgaaggcaaagaatcaatcgcacaagttgcttcaatctccgctgcagacgaagaagtcggaagcctgatcgctgaagcaatggagcgcgtcggcaacgacggtgttatcacgattgaagaatccaaaggattcacaacagagcttgaagtggttgaaggtatgcagttcgaccgcggatatgcgtctccttacatggtgacggattccgataagatggaagcggttcttgagaatccgtacatcttagtaacagacaaaaaaatcacaaacattcaagaaatcctgccggtgcttgagcaagtcgtgcaacaaggcaaaccgttgcttctgattgctgaagacgttgaaggtgaagctcttgcaacattggttgtcaacaagcttcgcggaacattcaacgcagtggctgttaaagcgcctggattcggcgaccgccgcaaagcgatgctcgaagacatctctatcctgacaggcgccgaagtgatcacagaagatttaggtcttgaccttaaatcaactcaaatcaatcaattgggacgcgcttctaaagttgttgttacaaaagaaaacacaacaattgttgaaggtgcgggagatacagagcaaatcgcggcacgcgtcaaccaaatccgcgctcaagttgaagaaacaacttctgagttcgataaagaaaaattacaagaacgccttgctaagcttgcaggcggcgtagctgtcatcaaagtcggagctgcgactgaaacagaattgaaagaacgcaagcttcgcatcgaagacgccctgaactctactcgcgctgcggtagaagaaggaatcgtatccggcggtggtacagctcttgtcaatgtttacaataaagtagctgcccttgaagctgaaggcgacgaactgactggtatcaacatcgttcttcgcgctcttgaagaaccaatccgtcaaatcgcgcacaacgcgggtcttgaaggatctgtcatcgttgagcgcctgaaaaatgaagaaatcggcgtcggctacaacgctgcaacaggcgaatgggtgaacatgatcgacaaaggtatcgttgaccctacaaaagtaacacgctcagctctgcaaaacgcagcatctgtagcggctatgttcctgacaactgaagcagttgttgccgacaaaccggaagaaaacaaaggcggcgcaggaatgcctgacatgggcggcatgggcggcatgggcggcatgatgtaa

SEQ ID NO: 23 - DNA, 1197 bp, Bacillus licheniformis
  source 1..1197: mol_type = genomic DNA
gtgaagaataaatggctttcttttttttcaggaaagatccagcttaagataacgggaaaagggatcgaacggttattaaatgaatgcaccaggcgcaacatcccgatgtttaatgtaaagaaaaagaaagacgccgtctttctttatattccgctttctgatgtacatgccttccggaaggtcatcagaggcttcgactgcaagtgcaggttcatcaaacgaaaagggtttcctttcctcgtgcagaagtctaaacggaatagcggcttcacttttggagttgctgcattttttatcatcatgttcctattgtccaacatgctttggaaaattgatattacaggagccaatccagagacagaacatcaaatcagacagcaattggatcaaatcggcgtcaaaaaaggccgctttcagttttcaatgctgaccccggaaaaaattcagcaggcgctcacaaagcgggtcgaaaacatcacttgggtgggcattgagttaaacggtaccgcccttcacatgaaagtcgttgaaaagaatgaacctgacaaagaaaaatatatcggtccgaggcacatcgtcgccaaaaaaggggcgaccatctcgaaaatgttcgtggaaaaaggcgagccgctcgtcacggtgaaccagcacgttgaaaaagggcaaatgctcgtttccgggctgatcggaagcgaagaggaaaagcaaaaagtcggagcaaaagggaaaatctatggtgaaacctggtacaagtcaacagtaacggttcctcttgagacatcatttgacgtttttacgggtaaagtaaggacaagtcacaagctatccctcggatcattttccgtgccgatctggggcttttcatttaaaaaagaagacttctcgcgcccgaagacggagaccgaaaaacactcgctgcattttatgaattttaagcttcctgtcgcttatgaaaaggagcatatgagggagagcgaacaaatcaaaagggtgtactcgaaaaaagaagcagttcttgaaggaatcgaaatgggaaaaagagacatcaggaaaaaaatcggcagcgacgggaacattatcagtgaaaaagttttgcacgaaacgagcgagaatggtaaagttaaattgatcatcctttaccaggttattgaagacattgttcaaacaacaccaattgttcaggagactaaagaatga

SEQ ID NO: 24 - DNA, 561 bp, Bacillus licheniformis
  source 1..561: mol_type = genomic DNA
atgaacagcaaatcacgattgacgcctgaaatgtggcgggcaattacggaaaacgattccgcctatgacggagttttttattacgcggtcaaaacgaccggcatattttgccgcccatcctgcaaatcgagagttccgcaaatcgacaatgtgcagatctttttcaatgcaaaagatgctttatcagaagggttccgcccctgcaaacgctgcaatcccgccggggcgctgctgccggatgaagagctggcacagcgggtagtgcaaatcatcgagaaatcttatcgcgatccgctgtctctgcaagctttggctgacaggtgccatatcagcccttttcacctgcagcggacatttaaacgaatcaaaggcgtctcgccggcagaatacatcctgcagaaaaggattgagaaagcggtcgatttgcttgctcattcagaacgatcgatcgcagaaatcgcttcaatggtaggcattgcgaatgcggaatattttgcctctttgtttaaaaagaagactgggcaatcgccgacgtcgtaccggcaaatgaaacggaggtaa

SEQ ID NO: 25 - DNA, 1552 bp, Priestia megaterium
  source 1..1552: mol_type = genomic DNA
tcttcggagagtttgatcctggctcaggatgaacgctggcggcgtgcctaatacatgcaagtcgagcgaactgattagaagcttgcttctatgacgttagcggcggacgggtgagtaacacgtgggcaacctgcctgtaagactgggataacttcgggaaaccgaagctaataccggatacgatcttctccttcatgggagatgattgaaagatggtttcggctatcacttacagatgggcccgcggtgcattagctagttggtgaggtaacggctcaccaaggcaacgatgcatagccgacctgagagggtgatcggccacactgggactgagacacggcccagactcctacgggaggcagcagtagggaatcttccgcaatggacgaaagtctgacggagcaacgccgcgtgagtgatgaaggctttcgggtcgtaaaactctgttgttagggaagaacaagtacgagagtaactgctcgtaccttgacggtacctaaccagaaagccacggctaactacgtgccagcagccgcggtaatacgtaggtggcaagcgttatccggaattattgggcgtaaagcgcgcgcaggcggtttcttaagtctgatgtgaaagcccacggctcaaccgtggagggtcattggaaactggggaacttgagtgcagaagagaaaagcggaattccacgtgtagcggtgaaatgcgtagagatgtggaggaacaccagtggcgaaggcggctttttggtctgtaactgacgctgaggcgcgaaagcgtggggagcaaacaggattagataccctggtagtccacgccgtaaacgatgagtgctaagtgttagagggtttccgccctttagtgctgcagctaacgcattaagcactccgcctggggagtacggtcgcaagactgaaactcaaaggaattgacgggggcccgcacaagcggtggagcatgtggtttaattcgaagcaacgcgaagaaccttaccaggtcttgacatcctctgacaactctagagatagagcgttccccttcgggggacagagtgacaggtggtgcatggttgtcgtcagctcgtgtcgtgagatgttgggttaagtcccgcaacgagcgcaacccttgatcttagttgccagcattcagttgggcactctaaggtgactgccggtgacaaaccggaggaaggtggggatgacgtcaaatcatcatgccccttatgacctgggctacacacgtgctacaatggatggtacaaagggctgcaagaccgcgaggtcaagccaatcccataaaaccattctcagttcggattgtaggctgcaactcgcctacatgaagctggaatcgctagtaatcgcggatcagcatgccgcggtgaatacgttcccgggccttgtacacaccgcccgtcacaccacgagagtttgtaacacccgaagtcggtggagtaaccgtaaggagctagccgcctaaggtgggacagatgattggggtgaagtcgtaacaaggtagccgtatcggaaggtgcggctggatcacctccttt

SEQ ID NO: 26 - DNA, 3564 bp, Priestia megaterium
  source 1..3564: mol_type = genomic DNA
ttgacaggtcaactagttcagtatggacgccaccgccaacgcagaagttatgctcgtattagtgaagttttagagttaccgaacttaatcgagattcaaacggcttcataccaatggtttttagatgaaggtttacgagaaatgttccaagatatttctccaattgatgattttacaggtaacttatcactagaatttattgattacagcttaggtgagccaaagtattcagtaggagagtctaaagaacgtgatgtaacttatgcagcacctcttcgtgttaaggtgcggttaattaataaagaaacaggtgaagtaaaagaccaagatgtgttcatgggagatttcccattgatgaccgaaacaggtacctttgtaattaacggtgctgagcgtgttatcgtatcacagttggttcgttcaccaagtgtttactatagtggaaagcttgataaaaacggtaaaaaaggatatacagcaactgttatccctaaccgtggtgcatggctagaatatgaaactgatgcaaaagatgtagtatacgtgcgtattgatcgtactcgtaaactgccagtaacagtgctgttacgcgcgctaggtttcggttctgaccaagagattatcgatttaatcggtgataatgaatacatccgtaatacgcttgaaaaagataatacggaaacaacggaaaaagcgctattagaaatctatgagcgtttacgtccgggtgaaccaccgacagttgagaatgcgaagtctctattagtatctcgcttctttgatccaaaacgatatgacttagcgaacgtaggtcgctataaaattaataaaaagcttcatatcaaacatcgcttatttaatcaaaagctagctgaaacattagttgatcctgaaacaggtgaaattattgcagaaaaaggcgcaatgattgaccgccgtctgctagatcgcttgattccgatgcttgaaggtggagtaaacttcaaaacttatagtccggttggtggagtagtagaagacgatgttacattacaatctattaagatttatgcgccaaatgatccagaaggtgaaaaaatcatcactgtatcaggtaacgcatatgtaacagaagaagttaaaaatatcacacctgctgatattttagcatcaatcagttacttctttaacttgcttcatcaagtaggagacacagatgatatcgaccacttaggtaaccgtcgtctgcgttctgtaggtgaattgttacaaaaccaattccgtatcggtttatctcgtatggaacgtgttgttcgtgaaagaatgtcaattcaagacacgaatacaatcacacctcaacaattaattaatattcgcccagttattgcggcgattaaagagttctttggaagttctcaattatcacagttcatggatcaaacgaatccattaggcgaattgacgcacaaacgtcgtctttcagctctaggacctggtggtttaacgcgtgagcgcgctggtttcgaagtgcgtgacgttcactactcccactatggccgtatgtgtccgattgaaacaccagagggtccgaatatcgggttaatcaactcactatcttcttatgcaaaagtaaacaaattcggtttcatcgaaacaccttaccgtcgtatcgatcctgaaacaggtaaagtgacagagcgaattgactacttaacagctgatgaagaagataactatgttgtagcccaagcgaacgctcgtctaggtgatgatggttcattcttagatgaaaatgtcgttgcacgtttccgtggagaaaacacggttatccgtcgcgatcgtttagactatatggatgtatcaccaaaacaagttgtatctgccgctacagcatgtatcccattcttagagaacgatgactctaaccgtgcattaatgggtgcgaacatgcaacgtcaagcagtacctttattaaatcctgaagcaccaatcgtaggtacaggtatggaatacgtatctggtaaagactctggtgcagccgtgatttgtaaatatcctggcgttgtagagcgcgtagaagcaaaacaaatttttgttcgccgctatgaagaagtagacggacaaaaagttaaaggtaacttagatcaatacaaattattaaaatttgttcgttctaaccaaggtacttgttacaaccagcgtccgattgtttcagttggcgacgaagtagtaaaaggtgagatcttagccgacggtccttcaatggaaaaaggtgagcttgctttaggacgaaacgtaatggttggtttcatgacatgggatggttacaactatgaggatgccatcatcatgagtgaacgccttgtgaaagacgatgtatatacgtctgttcatattgaagaatatgaatctgagtctcgtgatacgaagcttggacctgaagaaattacgcgtgacattccaaacgtaggtgaagatgcgcttcgcaacttagatgagcgtggaatcatccgcattggtgcagaagtaaaagacggagatcttttagttggtaaagtaacgccaaaaggtgtaacagaactaacagctgaagaacgtcttctacacgctattttcggtgaaaaagcgcgtgaagttcgtgatacttctcttcgtgtaccgcacggcggcggtggaatcattcttgatgttaaagtcttcaaccgtgaagatggcgacgaattaccaccaggtgtaaaccaattagtccgtgtatatattgttcagaagcgtaaaatttctgaaggtgacaaaatggccggtcgtcacggtaacaaaggtgtaatttcacgtattttacctgaagaagatatgccttacctaccagacggtacgccaattgacatcatgttaaacccattaggggtaccatctcgtatgaacatcggtcaggtgctagagcttcatttaggtatggctgctcgtaagcttggcattcacgttgcgtctccagtatttgatggtgcgcgtgaggaagatgtttgggcaacaatcgaagaagctggcatgtctcgtgatgctaaaacagttctatatgatggtcgaacaggtgaaccattcgataaccgtgtatcagtaggaatcatgtacatgatcaaacttgctcacatggtagacgataaacttcacgctcgttctactggaccatactcacttgttacacaacaaccacttggtggtaaagcgcagttcggtggacagcgttttggtgagatggaggtatgggcacttgaagcatacggtgctgcttacacattacaagagatcttaacagtgaaatcagatgacgtagtaggtcgtgtgaaaacatacgaagcaattgttaaaggtgaaaacattccagaacctggcatacctgaatcgttcaaagtattaattaaagaactacaaagtttaggtatggatgtgaagatgctttctgctgacgagcaagaaattgatatcatggactcagaagaggaccatgagcaaccaacagaatcaattattgcagataacgaagaaagcctttctgaaggacaaaaagatcctgtcacaaaagagtaa

SEQ ID NO: 27 - DNA, 1923 bp, Priestia megaterium
  source 1..1923: mol_type = genomic DNA
ttgacgatggaacaaaaagaagtacaagcatatgaagctgatcagatacaagtattagaaggattagaagctgttcgtaaacgtccggggatgtatattggatcgacgagcgcaaagggtctacatcatcttgtatgggaaattgtagataatagtattgatgaagcgctggccggctattgcgatgaaattaatgttattatcgaaaaggataatagtattacagtcaaagataacggtcgtggaattccggttggtattcaagaaaaaatgggcagacctgccgttgaagttatcttaacggttcttcatgccggaggtaaatttggcggcggcggctataaagtatctggtggattacacggtgtaggtgcctcagttgttaatgcactttctacctctttggaagtgcacgtacatcgtgacggtaaagttcattatcaaaaatatgaacgaggtgtaccggctgctgacttaaaagtagttggagaaacagataaaacaggtactgttattcaattccgtccagacggtgaaatttttacagaaacgcttgaatacgattttgatacgttagctaatcgtctgcgtgagttagctttcttaaatcgcggcattaaaattacgattgaagacaaacgtgaagaagataaaagacgtgagtatcactatgaaggcggaattaagtcttacgttgaacacttaaaccgttcgaaagaagtgattcacgaagagccaatctatattgaaggtaatcgagacaacatttctgtagaaattgctattcaatataacgatagctatacaagtaatttatattcttttgcaaacaatattcacacatatgaaggtggaacgcacgaagcaggatttaaaacagcgttaacgcgtgtaattaacgactatgcacgtaaaaacagcgtatttaaagacagtgacgccaatctaacaggtgaagatgttcgtgaaggaattacagctatcatctctattaagcacccagatccgcagttcgaaggacaaacaaaaacaaagctgggaaatagtgaagcaagaacaattactgactctgtgtttgcagaacacttagaaacttacttgctagagaaccctattgtggcgaaaaaggtaattgaaaaaggtttaatggctgcaagagcaagaatggcagctaaaaaagctcgtgagcttacacgccgtaaaagcgcgcttgaaatttcaaacttaccgggtaaattagcagattgttcatcaaaagatccttctattagcgaactctatgtagtagagggtgactctgccggaggttcagctaagcagggaagaagccgtcatttccaagctattttgcctttacgtggtaaaattatcaacgtagagaaagcgcgtttagataaaattttatctaataacgaaattcgtacaatcattaccgctctaggaacgggtattggtgacgattttgatatttcgaaagcccgctaccataaaattgtgattatgacagatgcagacgtagacggtgcgcatattcgtacgcttcttctaacgttcttctatcgctatatgagacagattattgagcacggatatgtgtacattgctcagccgcctctttacaaagtttcacaaggtaaaaaagtggagtacgcgtacaacgatcgtcaattagaagaggtattagcttctttccctgaaggcgcaaaaccaaaccttcagcgttacaaaggtttaggagagatgaatcctgaacaattatgggaaacaacaatggatccagagttccgtacccttcttcaggtgaacttgcaagatgcaattgaagctgatgagacatttgaaattttaatgggcgacaaagtagaaccacgccgtaatttcattgaagaaaatgctcagtacgtaaaaaatcttgatatttaa

SEQ ID NO: 28 - DNA, 1632 bp, Priestia megaterium
  source 1..1632: mol_type = genomic DNA
atggcaaaagacattaaatttagcgaagaagcacgtcgcgcaatgctacgtggtgtagatacattagcaaatgcggtaaaagtaacgcttggaccaaaaggtcgtaacgttgtattagaaaagaaattcggttcaccgcttattacaaatgacggtgtaacaattgcaaaagaaatcgaattagaagacgcatttgaaaatatgggtgctaaattagtagctgaagttgctagcaaaacaaacgacgttgctggtgacggtacaactactgcaacagttttagcgcaagcaatgatcagagaaggccttaaaaacgtaacggctggtgctaacccaatgggtatccgtaaaggtatggaaaaagcagtagctgtagcggttgaagaactaaaagcaatctctaaaccaattcaaggtaaagattcaattgctcaagtagcggctatctcagcggctgacgaagaagtaggtcaactaatcgctgaagcaatggagcgcgttggtaacgacggcgttatcacacttgaagagtcaaaaggtttcacaactgaattagaagtggtagaaggtatgcagtttgaccgtggatatgcatctccttacatggtaactgattcagataaaatggaagctgtattagatgacccgtacatcttaattacagacaaaaaaattggtaacattcaagaaatcttaccggtattagagcaagttgttcaacaaggcaagcctctattaatcatcgctgaagacgtagaaggcgaagctttagcaacattagttgtgaacaaacttcgcggtacatttacagctgtagctgttaaagctcctggtttcggtgatcgtcgtaaagcaatgctacaagacgttgcgatcttaacaggcggagaagtaatcactgaagagcttggtcttgacctgaaaacagcaagcatcgaccaattaggtcgcgcttctaaaattgttgtaacaaaagaaaatacaacagttgtaaacggtgcaggaaacgcagaagatatcctagcacgcgtaaaccaaatcaaagctcagcttgaagaaacaacttcagagtttgaccgcgaaaaattacaagagcgcttagcaaaacttgctggtggcgtagctgtaattaaagttggtgcggcaactgaaactgagttaaaagaacgtaaattacgtattgaagatgcattaaactctacgcgcgctgcggttgaagaaggtatcgtagctggtggtggtactgcattagtaaatatctataataaagtagcaagcatcgaagctgacggtgacactgctacaggtatcaacatcgtattacgtgcgattgaagagcctgtacgtcaaatcgctcacaacgctggtttagaaggatccgtaatcgttgagcgtctaaaaggcgaagcagttggaactggatttaacgctgcaactggcgagtgggtaaatatgctagacactggtatcgttgacccaacaaaagtaacgcgttcagctcttcaaaatgcttcttctgtagcagctatgttcttaacaactgaagcagttgttgctgacaagccagaagaaaacgcagctcctgcaatgcctgacatgggcggcatgggtggaatgggcggcatgatgtaa

SEQ ID NO: 29 - DNA, 1188 bp, Priestia megaterium
  source 1..1188: mol_type = genomic DNA
atgaagaatggatggacaaactttgttattggtaccgtacgtattcgaattgttggaaaaggaattgaacgttttttaaataattgtgtgagacaacagattatgatttcgaatgtccataaagttgacggtcagctagcgacagcaacgatattattgaaagatgtaaagaaaattcgtatactaattcgcaacgcagattgtaaaatttattttataagaggcagaggttttccttttttaacaaaacgagtgatcaaaaatagtgggtttgctttgggttttctttctttttttattattcttggtttgctttccaacatggtgtggaaagtggaaattagcggtgcagaaccacaaacagaacatcaaatgactaagcagcttgccaaaataggtgtaaaaagaggggagtttcaatttctgttagagagtcctgaaaaaattcagcgctatttaacggataatatgaacaatattacctgggtgggagtagaagtgcgcggcacttcttatcacttccaagtggttgaaaaaaatgagcccaagcctcagcaaaaaacaccttaccaacatttaattgctaaaaagaaagccattattacgaatttgtttgtcgaaaaaggacaacctttagtcaaggttaatgattttgtcaatgaaggcgaggtcctagtttccggtattattggaaacgaaaaaaataaaaaagtagtagctgctaaagggaaagtctatggtgaaacatggtataagtctgaggtggaagtgcctttaaaaactgattttcaggtattaacgggtaatggatatacgaagcactatttagattttcaagcttttaaaatgcctctttgggcttttaacaaagaaaaatacggctcaaaggtgacagaaaaagtggagcatccactctatttttttaaatggaaattacctctgttgtatgagaaagttgctgtacgagaagaacagaactcgcagcgcgtctattctaaacaagaggcggtggaaaaagctttggaaattggtagaaaaaaattactatcaactttaggtgaggatgctaaaataaaaggtgaaaaagttttgcaccaagaacaggacaatggtaaagttagattatcaatacattaccaagttatagaaaatattgcgaacactcaaccaattattcaaggagattga